European Patent Application EP 4 137 161 A1, published February 22, 2023. Title: METHOD AND DRUG FOR TREATING HURLER SYNDROME. Applicant: EdiGene Inc. The sequence listing filed with the application follows.

SEQUENCE LISTING (83 sequences)

SEQ ID NO: 1 - DNA, 20 bp, Artificial sequence
  hIDUA-F1
cgcttccaggtcaacaacac

SEQ ID NO: 2 - DNA, 19 bp, Artificial sequence
  hIDUA-R1
ctcgcgtagatcagcaccg

SEQ ID NO: 3 - RNA, 111 nt, Artificial sequence
  arRNA
gacgcccaccgugugguugcuguccaggacggucccggccugcgacacuucggcccagagcugcuccucauccagcagcgccagcagccccauggccgugagcaccggcuu

SEQ ID NO: 4 - RNA, 111 nt, Artificial sequence
  arRNA
gacgcccaccgugugguugcuguccaggacggucccggccugcgacacuucggcccagagcugcuccucaucugcggggcgggggggggccgucgccgcguggggucguug

SEQ ID NO: 5 - RNA, 111 nt, Artificial sequence
  arRNA
uaccgcuacagccacgcugauuucagcuauaccugcccgguauaaagggacguucacaccgcgauguucucugcuggggaauugcgcgauauucaggauuaaaagaagugc

SEQ ID NO: 6 - RNA, 91 nt, Artificial sequence
  arRNA
uaauccugaauaucgcgcaauuccccagcagagaacaucgcggugugaacgucccuuuauaccgggcagguauagcugaaaucagcguggc

SEQ ID NO: 7 - RNA, 71 nt, Artificial sequence
  arRNA
uuucagcuauaccugcccgguauaaagggacguucacaccgcgauguucucugcuggggaauugcgcgaua

SEQ ID NO: 8 - RNA, 51 nt, Artificial sequence
  arRNA
uuccccagcagagaacaucgcggugugaacgucccuuuauaccgggcaggu

SEQ ID NO: 9 - RNA, 91 nt, Artificial sequence
  arRNA
gugugguugcuguccaggacggucccggccugcgacacuucggcccagagcugcuccucaucugcggggcgggggggggccgucgccgcgu

SEQ ID NO: 10 - RNA, 71 nt, Artificial sequence
  arRNA
uguccaggacggucccggccugcgacacuucggcccagagcugcuccucaucugcggggcgggggggggcc

SEQ ID NO: 11 - RNA, 51 nt, Artificial sequence
  arRNA
ggucccggccugcgacacuucggcccagagcugcuccucaucugcggggcg

SEQ ID NO: 12 - RNA, 101 nt, Artificial sequence
  arRNA
gacgcccaccgugugguugcuguccaggacggucccggccugcgacacuucggcccagagcugcuccucaucugcggggcgggggggggccgucgccgcgu

SEQ ID NO: 13 - RNA, 91 nt, Artificial sequence
  arRNA
gacgcccaccgugugguugcuguccaggacggucccggccugcgacacuucggcccagagcugcuccucaucugcggggcgggggggggcc

SEQ ID NO: 14 - RNA, 81 nt, Artificial sequence
  arRNA
gacgcccaccgugugguugcuguccaggacggucccggccugcgacacuucggcccagagcugcuccucaucugcggggcg

SEQ ID NO: 15 - RNA, 71 nt, Artificial sequence
  arRNA
gacgcccaccgugugguugcuguccaggacggucccggccugcgacacuucggcccagagcugcuccucau

SEQ ID NO: 16 - RNA, 61 nt, Artificial sequence
  arRNA
gacgcccaccgugugguugcuguccaggacggucccggccugcgacacuucggcccagagc

SEQ ID NO: 17 - RNA, 101 nt, Artificial sequence
  arRNA
gugugguugcuguccaggacggucccggccugcgacacuucggcccagagcugcuccucaucugcggggcgggggggggccgucgccgcguggggucguug

SEQ ID NO: 18 - RNA, 91 nt, Artificial sequence
  arRNA
uguccaggacggucccggccugcgacacuucggcccagagcugcuccucaucugcggggcgggggggggccgucgccgcguggggucguug

SEQ ID NO: 19 - RNA, 81 nt, Artificial sequence
  arRNA
ggucccggccugcgacacuucggcccagagcugcuccucaucugcggggcgggggggggccgucgccgcguggggucguug

SEQ ID NO: 20 - RNA, 71 nt, Artificial sequence
  arRNA
ugcgacacuucggcccagagcugcuccucaucugcggggcgggggggggccgucgccgcguggggucguug

SEQ ID NO: 21 - RNA, 61 nt, Artificial sequence
  arRNA
cggcccagagcugcuccucaucugcggggcgggggggggccgucgccgcguggggucguug

SEQ ID NO: 22 - RNA, 80 nt, Artificial sequence
  arRNA
gacgcccaccgugugguugcuguccaggacggucccggccugcgacacuucggcccagagcugcuccucaucugcggggc

SEQ ID NO: 23 - RNA, 79 nt, Artificial sequence
  arRNA
gacgcccaccgugugguugcuguccaggacggucccggccugcgacacuucggcccagagcugcuccucaucugcgggg

SEQ ID NO: 24 - RNA, 78 nt, Artificial sequence
  arRNA
gacgcccaccgugugguugcuguccaggacggucccggccugcgacacuucggcccagagcugcuccucaucugcggg

SEQ ID NO: 25 - RNA, 77 nt, Artificial sequence
  arRNA
gacgcccaccgugugguugcuguccaggacggucccggccugcgacacuucggcccagagcugcuccucaucugcgg

SEQ ID NO: 26 - RNA, 76 nt, Artificial sequence
  arRNA
gacgcccaccgugugguugcuguccaggacggucccggccugcgacacuucggcccagagcugcuccucaucugcg

SEQ ID NO: 27 - RNA, 75 nt, Artificial sequence
  arRNA
gacgcccaccgugugguugcuguccaggacggucccggccugcgacacuucggcccagagcugcuccucaucugc

SEQ ID NO: 28 - RNA, 74 nt, Artificial sequence
  arRNA
gacgcccaccgugugguugcuguccaggacggucccggccugcgacacuucggcccagagcugcuccucaucug

SEQ ID NO: 29 - RNA, 73 nt, Artificial sequence
  arRNA
gacgcccaccgugugguugcuguccaggacggucccggccugcgacacuucggcccagagcugcuccucaucu

SEQ ID NO: 30 - RNA, 72 nt, Artificial sequence
  arRNA
gacgcccaccgugugguugcuguccaggacggucccggccugcgacacuucggcccagagcugcuccucauc

SEQ ID NO: 31 - RNA, 70 nt, Artificial sequence
  arRNA
gacgcccaccgugugguugcuguccaggacggucccggccugcgacacuucggcccagagcugcuccuca

SEQ ID NO: 32 - RNA, 69 nt, Artificial sequence
  arRNA
gacgcccaccgugugguugcuguccaggacggucccggccugcgacacuucggcccagagcugcuccuc

SEQ ID NO: 33 - RNA, 68 nt, Artificial sequence
  arRNA
gacgcccaccgugugguugcuguccaggacggucccggccugcgacacuucggcccagagcugcuccu

SEQ ID NO: 34 - RNA, 67 nt, Artificial sequence
  arRNA
gacgcccaccgugugguugcuguccaggacggucccggccugcgacacuucggcccagagcugcucc

SEQ ID NO: 35 - RNA, 66 nt, Artificial sequence
  arRNA
gacgcccaccgugugguugcuguccaggacggucccggccugcgacacuucggcccagagcugcuc

SEQ ID NO: 36 - RNA, 65 nt, Artificial sequence
  arRNA
gacgcccaccgugugguugcuguccaggacggucccggccugcgacacuucggcccagagcugcu

SEQ ID NO: 37 - RNA, 64 nt, Artificial sequence
  arRNA
gacgcccaccgugugguugcuguccaggacggucccggccugcgacacuucggcccagagcugc

SEQ ID NO: 38 - RNA, 63 nt, Artificial sequence
  arRNA
gacgcccaccgugugguugcuguccaggacggucccggccugcgacacuucggcccagagcug

SEQ ID NO: 39 - RNA, 62 nt, Artificial sequence
  arRNA
gacgcccaccgugugguugcuguccaggacggucccggccugcgacacuucggcccagagcu

SEQ ID NO: 40 - RNA, 70 nt, Artificial sequence
  arRNA
uaccgcuacagccacgcugauuucagcuauaccugcccgguauaaagggacguucacaccgcgauguucu

SEQ ID NO: 41 - RNA, 66 nt, Artificial sequence
  arRNA
uaccgcuacagccacgcugauuucagcuauaccugcccgguauaaagggacguucacaccgcgaug

SEQ ID NO: 42 - RNA, 71 nt, Artificial sequence
  arRNA
ccaccgugugguugcuguccaggacggucccggccugcgacacuucggcccagagcugcuccucaucugcg

SEQ ID NO: 43 - RNA, 66 nt, Artificial sequence
  arRNA
gugugguugcuguccaggacggucccggccugcgacacuucggcccagagcugcuccucaucugcg

SEQ ID NO: 44 - RNA, 61 nt, Artificial sequence
  arRNA
guugcuguccaggacggucccggccugcgacacuucggcccagagcugcuccucaucugcg

SEQ ID NO: 45 - RNA, 56 nt, Artificial sequence
  arRNA
uguccaggacggucccggccugcgacacuucggcccagagcugcuccucaucugcg

SEQ ID NO: 46 - RNA, 66 nt, Artificial sequence
  arRNA
ccaccgugugguugcuguccaggacggucccggccugcgacacuucggcccagagcugcuccucau

SEQ ID NO: 47 - RNA, 61 nt, Artificial sequence
  arRNA
gugugguugcuguccaggacggucccggccugcgacacuucggcccagagcugcuccucau

SEQ ID NO: 48 - RNA, 56 nt, Artificial sequence
  arRNA
guugcuguccaggacggucccggccugcgacacuucggcccagagcugcuccucau

SEQ ID NO: 49 - RNA, 51 nt, Artificial sequence
  arRNA
uguccaggacggucccggccugcgacacuucggcccagagcugcuccucau

SEQ ID NO: 50 - RNA, 67 nt, Artificial sequence
  arRNA
acgcccaccgugugguugcuguccaggacggucccggccugcgacacuucggcccagagcugcuccu

SEQ ID NO: 51 - RNA, 67 nt, Artificial sequence
  arRNA
cgcccaccgugugguugcuguccaggacggucccggccugcgacacuucggcccagagcugcuccuc

SEQ ID NO: 52 - RNA, 67 nt, Artificial sequence
  arRNA
gcccaccgugugguugcuguccaggacggucccggccugcgacacuucggcccagagcugcuccuca

SEQ ID NO: 53 - RNA, 67 nt, Artificial sequence
  arRNA
cccaccgugugguugcuguccaggacggucccggccugcgacacuucggcccagagcugcuccucau

SEQ ID NO: 54 - RNA, 67 nt, Artificial sequence
  arRNA
ccaccgugugguugcuguccaggacggucccggccugcgacacuucggcccagagcugcuccucauc

SEQ ID NO: 55 - RNA, 67 nt, Artificial sequence
  arRNA
caccgugugguugcuguccaggacggucccggccugcgacacuucggcccagagcugcuccucaucu

SEQ ID NO: 56 - RNA, 67 nt, Artificial sequence
  arRNA
accgugugguugcuguccaggacggucccggccugcgacacuucggcccagagcugcuccucaucug

SEQ ID NO: 57 - RNA, 67 nt, Artificial sequence
  arRNA
ccgugugguugcuguccaggacggucccggccugcgacacuucggcccagagcugcuccucaucugc

SEQ ID NO: 58 - RNA, 67 nt, Artificial sequence
  arRNA
cgugugguugcuguccaggacggucccggccugcgacacuucggcccagagcugcuccucaucugcg

SEQ ID NO: 59 - RNA, 67 nt, Artificial sequence
  arRNA
gugugguugcuguccaggacggucccggccugcgacacuucggcccagagcugcuccucaucugcgg

SEQ ID NO: 60 - RNA, 67 nt, Artificial sequence
  arRNA
ugugguugcuguccaggacggucccggccugcgacacuucggcccagagcugcuccucaucugcggg

SEQ ID NO: 61 - RNA, 67 nt, Artificial sequence
  arRNA
gugguugcuguccaggacggucccggccugcgacacuucggcccagagcugcuccucaucugcgggg

SEQ ID NO: 62 - RNA, 70 nt, Artificial sequence
  arRNA
acgcccaccgugugguugcuguccaggacggucccggccugcgacacuucggcccagagcugcuccucau

SEQ ID NO: 63 - RNA, 70 nt, Artificial sequence
  arRNA
cgcccaccgugugguugcuguccaggacggucccggccugcgacacuucggcccagagcugcuccucauc

SEQ ID NO: 64 - RNA, 70 nt, Artificial sequence
  arRNA
gcccaccgugugguugcuguccaggacggucccggccugcgacacuucggcccagagcugcuccucaucu

SEQ ID NO: 65 - RNA, 70 nt, Artificial sequence
  arRNA
cccaccgugugguugcuguccaggacggucccggccugcgacacuucggcccagagcugcuccucaucug

SEQ ID NO: 66 - RNA, 70 nt, Artificial sequence
  arRNA
ccaccgugugguugcuguccaggacggucccggccugcgacacuucggcccagagcugcuccucaucugc

SEQ ID NO: 67 - RNA, 70 nt, Artificial sequence
  arRNA
caccgugugguugcuguccaggacggucccggccugcgacacuucggcccagagcugcuccucaucugcg

SEQ ID NO: 68 - RNA, 70 nt, Artificial sequence
  arRNA
accgugugguugcuguccaggacggucccggccugcgacacuucggcccagagcugcuccucaucugcgg

SEQ ID NO: 69 - RNA, 70 nt, Artificial sequence
  arRNA
ccgugugguugcuguccaggacggucccggccugcgacacuucggcccagagcugcuccucaucugcggg

SEQ ID NO: 70 - RNA, 70 nt, Artificial sequence
  arRNA
cgugugguugcuguccaggacggucccggccugcgacacuucggcccagagcugcuccucaucugcgggg

SEQ ID NO: 71 - RNA, 72 nt, Artificial sequence
  arRNA
acgcccaccgugugguugcuguccaggacggucccggccugcgacacuucggcccagagcugcuccucaucu

SEQ ID NO: 72 - RNA, 72 nt, Artificial sequence
  arRNA
cgcccaccgugugguugcuguccaggacggucccggccugcgacacuucggcccagagcugcuccucaucug

SEQ ID NO: 73 - RNA, 72 nt, Artificial sequence
  arRNA
gcccaccgugugguugcuguccaggacggucccggccugcgacacuucggcccagagcugcuccucaucugc

SEQ ID NO: 74 - RNA, 72 nt, Artificial sequence
  arRNA
cccaccgugugguugcuguccaggacggucccggccugcgacacuucggcccagagcugcuccucaucugcg

SEQ ID NO: 75 - RNA, 72 nt, Artificial sequence
  arRNA
ccaccgugugguugcuguccaggacggucccggccugcgacacuucggcccagagcugcuccucaucugcgg

SEQ ID NO: 76 - RNA, 72 nt, Artificial sequence
  arRNA
caccgugugguugcuguccaggacggucccggccugcgacacuucggcccagagcugcuccucaucugcggg

SEQ ID NO: 77 - RNA, 72 nt, Artificial sequence
  arRNA
accgugugguugcuguccaggacggucccggccugcgacacuucggcccagagcugcuccucaucugcgggg

SEQ ID NO: 78 - DNA, 20 bp, Artificial sequence
  hIDUA-62F
ccttcctgagctaccacccg

SEQ ID NO: 79 - DNA, 20 bp, Artificial sequence
  hIDUA-62R
ccagggctcgaactcggtag

SEQ ID NO: 80 - RNA, 70 nt, Artificial sequence
  arRNA
caccgugugguugcuguccaggacggucccggccugcgacacuucggcccagagccgcuccucaucugcg

SEQ ID NO: 81 - RNA, 50 nt, Artificial sequence
  arRNA
cuguccaggacggucccggccugcgacacuucggcccagagcugcuccuc

SEQ ID NO: 82 - DNA, 34 bp, Artificial sequence
  arRNA
gatgaggagcagctctgggccgaagtgtcgcagg

SEQ ID NO: 83 - DNA, 34 bp, Artificial sequence
  arRNA
gatgaggagcagctctaggccgaagtgtcgcagg